European Patent Application EP 4 722 232 A1, published April 8, 2026. Title: 使用时活化的单链多肽. Applicant: 妍诗美社（海南）医美健康科技有限公司. Application WO. The sequence listing filed with the application follows.

SEQUENCE LISTING (51 sequences)

SEQ ID NO: 1 - protein, 6 aa, synthetic construct
YRSRIV

SEQ ID NO: 2 - protein, 6 aa, synthetic construct
KHLYSN

SEQ ID NO: 3 - protein, 9 aa, synthetic construct
VSQVYPIVQ

SEQ ID NO: 4 - protein, 8 aa, synthetic construct
WEHDGIAE

SEQ ID NO: 5 - protein, 4 aa, synthetic construct
DDDK

SEQ ID NO: 6 - protein, 7 aa, synthetic construct
ENLYFQS

SEQ ID NO: 7-8 - skipped (2 entries)

SEQ ID NO: 9 - protein, 8 aa, synthetic construct
LEVLFQGP

SEQ ID NO: 10 - protein, 437 aa, synthetic construct
MPFVNKQFNYKDPVNGVDIAYIKIPNVGQMQPVKAFKIHNKIWVIPERDTFTNPEEGDLNPPPEAKQVPVSYYDSTYLSTDNEKDNYLKGVTKLFERIYSTDLGRMLLTSIVRGIPFWGGSTIDTELKVIDTNCINVIQPDGSYRSEELNLVIIGPSADIIQFECKSFGHEVLNLTRNGYGSTQYIRFSPDFTFGFEESLEVDTNPLLGAGKFATDPAVTLAHELIHAGHRLYGIAINPNRVFKVNTNAYYEMSGLEVSFEELRTFGGHDAKFIDSLQENEFRLYYYNKFKDIASTLNKAKSIVGTTASLQYMKNVFKEKYLLSEDTSGKFSVDKLKFDKLYKMLTEIYTEDNFVKFFKVLNRKTYLNFDKAVFKINIVPKVNYTIYDGFNLRNTNLAANFNGQNTEINNMNFTKLKNFTGLFEFYKLLCVRGIITS

SEQ ID NO: 11 - protein, 441 aa, synthetic construct
MPVTINNFNYNDPIDNNNIIMMEPPFARGTGRYYKAFKITDRIWIIPERYTFGYKPEDFNKSSGIFNRDVCEYYDPDYLNTNDKKNIFLQTMIKLFNRIKSKPLGEKLLEMIINGIPYLGDRRVPLEEFNTNIASVTVNKLISNPGEVERKKGIFANLIIFGPGPVLNENETIDIGIQNHFASREGFGGIMQMKFCPEYVSVFNNVQENKGASIFNRRGYFSDPALILMHELIHVLHGLYGIKVDDLPIVPNEKKFFMQSTDAIQAEELYTFGGQDPSIITPSTDKSIYDKVLQNFRGIVDRLNKVLVCISDPNININIYKNKFKDKYKFVEDSEGKYSIDVESFDKLYKSLMFGFTETNIAENYKIKTRASYFSDSLPPVKIKNLLDNEIYTIEEGFNISDKNMEKEYRGQNKAINKQAYEEISKEHLAVYKIQMCKSVR

SEQ ID NO: 12 - protein, 444 aa, synthetic construct
MPITINNFNYSDPVDNKNILYLDTHLNTLANEPEKAFRITGNIWVIPDRFSRNSNPNLNKPPRVTSPKSGYYDPNYLSTDSDKDTFLKEIIKLFKRINSREIGEELIYRLSTDIPFPGNNNTPINTFDFDVDFNSVDVKTRQGNNWVKTGSINPSVIITGPRENIIDPETSTFKLTNNTFAAQEGFGALSIISISPRFMLTYSNATNDVGEGRFSKSEFCMDPILILMHELNHAMHNLYGIAIPNDQTISSVTSNIFYSQYNVKLEYAEIYAFGGPTIDLIPKSARKYFEEKALDYYRSIAKRLNSITTANPSSFNKYIGEYKQKLIRKYRFVVESSGEVTVNRNKFVELYNELTQIFTEFNYAKIYNVQNRKIYLSNVYTPVTANILDDNVYDIQNGFNIPKSNLNVLFMGQNLSRNPALRKVNPENMLYLFTKFCHKAIDGR

SEQ ID NO: 13 - protein, 445 aa, synthetic construct
MTWPVKDFNYSDPVNDNDILYLRIPQNKLITTPVKAFMITQNIWVIPERFSSDTNPSLSKPPRPTSKYQSYYDPSYLSTDEQKDTFLKGIIKLFKRINERDIGKKLINYLVVGSPFMGDSSTPEDTFDFTRHTTNIAVEKFENGSWKVTNIITPSVLIFGPLPNILDYTASLTLQGQQSNPSFEGFGTLSILKVAPEFLLTFSDVTSNQSSAVLGKSIFCMDPVIALMHELTHSLHQLYGINIPSDKRIRPQVSEGFFSQDGPNVQFEELYTFGGLDVEIIPQIERSQLREKALGHYKDIAKRLNNINKTIPSSWISNIDKYKKIFSEKYNFDKDNTGNFVVNIDKFNSLYSDLTNVMSEVVYSSQYNVKNRTHYFSRHYLPVFANILDDNIYTIRDGFNLTNKGFNIENSGQNIERNPALQKLSSESVVDLFTKVCLRLTKNSR

SEQ ID NO: 14 - protein, 422 aa, synthetic construct
MPTINSFNYNDPVNNRTILYIKPGGCQQFYKSFNIMKNIWIIPERNVIGTIPQDFLPPTSLKNGDSSYYDPNYLQSDQEKDKFLKIVTKIFNRINDNLSGRILLEELSKANPYLGNDNTPDGDFIINDASAVPIQFSNGSQSILLPNVIIMGAEPDLFETNSSNISLRNNYMPSNHGFGSIAIVTFSPEYSFRFKDNSMNEFIQDPALTLMHELIHSLHGLYGAKGITTKYTITQKQNPLITNIRGTNIEEFLTFGGTDLNIITSAQSNDIYTNLLADYKKIASKLSKVQVSNPLLNPYKDVFEAKYGLDKDASGIYSVNINKFNDIFKKLYSFTEFDLATKFQVKCRQTYIGQYKYFKLSNLLNDSIYNISEGYNINNLKVNFRGQNANLNPRIITPITGRGLVKKIIRFCKNIVSVKGIR

SEQ ID NO: 15 - protein, 439 aa, synthetic construct
MPVAINSFNYNDPVNDDTILYMQIPYEEKSKKYYKAFEIMRNVWIIPERNTIGTNPSDFDPPASLKNGSSAYYDPNYLTTDAEKDRYLKTTIKLFKRINSNPAGKVLLQEISYAKPYLGNDHTPIDEFSPVTRTTSVNIKLSTNVESSMLLNLLVLGAGPDIFESCCYPVRKLIDPDVVYDPSNYGFGSINIVTFSPEYEYTFNDISGGHNSSTESFIADPAISLAHELIHALHGLYGARGVTYEETIEVKQAPLMIAEKPIRLEEFLTFGGQDLNIITSAMKEKIYNNLLANYEKIATRLSEVNSAPPEYDINEYKDYFQWKYGLDKNADGSYTVNENKFNEIYKKLYSFTESDLANKFKVKCRNTYFIKYEFLKVPNLLDDDIYTVSEGFNIGNLAVNNRGQSIKLNPKIIDSIPDKGLVEKIVKFCKSVIPRKGTK

SEQ ID NO: 16 - protein, 446 aa, synthetic construct
MPVNIKXFNYNDPINNDDIIMMEPFNDPGPGTYYKAFRIIDRIWIVPERFTYGFQPDQFNASTGVFSKDVYEYYDPTYLKTDAEKDKFLKTMIKLFNRINSKPSGQRLLDMIVDAIPYLGNASTPPDKFAANVANVSINKKIIQPGAEDQIKGLMTNLIIFGPGPVLSDNFTDSMIMNGHSPISEGFGARMMIRFCPSCLNVFNNVQENKDTSIFSRRAYFADPALTLMHELIHVLHGLYGIKISNLPITPNTKEFFMQHSDPVQAEELYTFGGHDPSVISPSTDMNIYNKALQNFQDIANRLNIVSSAQGSGIDISLYKQIYKNKYDFVEDPNGKYSVDKDKFDKLYKALMFGFTETNLAGEYGIKTRYSYFSEYLPPIKTEKLLDNTIYTQNEGFNIASKNLKTEFNGQNKAVNKEAYEEISLEHLVIYRIAMCKPVMYKNTGK

SEQ ID NO: 17 - protein, 848 aa, synthetic construct
ALNDLCIKVNNWDLFFSPSEDNFTNDLNKGEEITSDTNIEAAEENISLDLIQQYYLTFNFDNEPENISIENLSSDIIGQLELMPNIERFPNGKKYELDKYTMFHYLRAQEFEHGKSRIALTNSVNEALLNPSRVYTFFSSDYVKKVNKATEAAMFLGWVEQLVYDFTDETSEVSTTDKIADITIIIPYIGPALNIGNMLYKDDFVGALIFSGAVILLEFIPEIAIPVLGTFALVSYIANKVLTVQTIDNALSKRNEKWDEVYKYIVTNWLAKVNTQIDLIRKKMKEALENQAEATKAIINYQYNQYTEEEKNNINFNIDDLSSKLNESINKAMININKFLNQCSVSYLMNSMIPYGVKRLEDFDASLKDALLKYIYDNRGTLIGQVDRLKDKVNNTLSTDIPFQLSKYVDNQRLLSTFTEYINNIINTSILNLRYESNHLIDLSRYASKINIGSKVNFDPIDKNQIQLFNLESSKIEVILKNAIVYNSMYENFSTSFWIRIPKYFNSISLNNEYTIINCMENNSGWKVSLNYGEIIWTLQDTQEIKQRVVFKYSQMINISDYINRWIFVTITNNRLNNSKIYINGRLIDQKPISNLGNIHASNNIMFKLDGCRDTHRYIWIKYFNLFDKELNEKEIKDLYDNQSNSGILKDFWGDYLQYDKPYYMLNLYDPNKYVDVNNVGIRGYMYLKGPRGSVMTTNIYLNSSLYRGTKFIIKKYASGNKDNIVRNNDRVYINVVVKNKEYRLATNASQAGVEKILSALEIPDVGNLSQVVVMKSKNDQGITNKCKMNLQDNNGNDIGFIGFHQFNNIAKLVASNWYNRQIERSSRTLGCSWEFIPVDDGWGERPL

SEQ ID NO: 18 - protein, 850 aa, synthetic construct
APGICIDVDNEDLFFIADKNSFSDDLSKNERIEYDTQSNYIENRSSINELILDTNLISKIELPSENTESLTDFNVDVPVYEKQPAIKKIFTDENTIFQYLYSQTFPLDIRDISLTSSFDDALLFSNKVYSFFSMDYIKTANKVVEAGLFAGWVKQIVDDFVIEANKSSTMDKIADISLIVPYIGLALNVGNETAKGNFENAFEIAGASILLEFIPELLIPVVGAFLLESYIDNKNKIIKTIDNALTKRDEKWIDMYGLIVAQWLSTVNTQFYTIKEGMYKALNYQAQALEEIIKYKYNIYSEKEKSNINIDFNDINSKLNEGINQAIDNINDFINECSVSYLMKKMIPLAVEKLLDFDNTLKKNLLNYIDENKLYLIGSAEYEKSKVDKYLKTIIPFDLSMYTNNTILIEIFNKYNSEILNNIILNLRYRDNNLIDLSGYGANVEVYDGVKLNDKNQFKLTSSTNSEIRVTQNQNIIFNSMFLDFSVSFWIRIPKYKNDGIQNYIHNEYTIINCIKNNSGWKISIRGNRIIWTLTDINGKTKSVFFEYSIREDISDYINRWFFVTITNNSDNAKIYINGKLESNIDIKNIGEVIANGEIIFKLDGDIDRTQFIWMKYFSIFNTELSQSNIKEIYKIQSYSEYLKDFWGNPLMYNKEYYMFNAGNKNSYIKLKKDSSVGEILTRSKYNQNSNYINYRNLYIGEKFIIRRKSNSQSINDDIVRKEDYIYLDFFNSNREWRVYAYKDFKEEEKKLFLANIYDSNEFYKTIQIKEYDEQPTYSCQLLFKKDEESTDEIGLIGIHRFYESGIVLKDYKNYFCISKWYLKEVKRKPYNPNLGCNWQFIPKDEGWIE

SEQ ID NO: 19 - protein, 847 aa, synthetic construct
SLYNKTLDCRELLVKNTDLPFIGDISDVKTDIFLRKDINEETEVIYYPDNVSVDQVILSKNTSEHGQLDLLYPSIDSESEILPGENQVFYDNRTQNVDYLNSYYYLESQKLSDNVEDFTFTRSIEEALDNSAKVYTYFPTLANKVNAGVQGGLFLMWANDVVEDFTTNILRKDTLDKISDVSAIIPYIGPALNISNSVRRGNFTEAFAVTGVTILLEAFPEFTIPALGAFVIYSKVQERNEIIKTIDNCLEQRIKRWKDSYEWMMGTWLSRIITQFNNISYQMYDSLNYQAGAIKAKIDLEYKKYSGSDKENIKSQVENLKNSLDVKISEAMNNINKFIRECSVTYLFKNMLPKVIDELNEFDRNTKAKLINLIDSHNIILVGEVDKLKAKVNNSFQNTIPFNIFSYTNNSLLKDIINEYFNNINDSKILSLQNRKNTLVDTSGYNAEVSEEGDVQLNPIFPFDFKLGSSGEDRGKVIVTQNENIVYNSMYESFSISFWIRINKWVSNLPGYTIIDSVKNNSGWSIGIISNFLVFTLKQNEDSEQSINFSYDISNNAPGYNKWFFVTVTNNMMGNMKIYINGKLIDTIKVKELTGINFSKTITFEINKIPDTGLITSDSDNINMWIRDFYIFAKELDGKDINILFNSLQYTNVVKDYWGNDLRYNKEYYMVNIDYLNRYMYANSRQIVFNTRRNNNDFNEGYKIIIKRIRGNTNDTRVRGGDILYFDMTINNKAYNLFMKNETMYADNHSTEDIYAIGLREQTKDINDNIIFQIQPMNNTYYYASQIFKSNFNGENISGICSIGTYRFRLGGDWYRHNYLVPTVKQGNYASLLESTSTHWGFVPVSE

SEQ ID NO: 20 - protein, 831 aa, synthetic construct
DDSTCIKVKNNRLPYVADKDSISQEIFENKIITDETNVQNYSDKFSLDESILDGQVPINPEIVDPLLPNVNMEPLNLPGEEIVFYDDITKYVDYLNSYYYLESQKLSNNVENITLTTSVEEALGYSNKIYTFLPSLAEKVNKGVQAGLFLNWANEVVEDFTTNIMKKDTLDKISDVSVIIPYIGPALNIGNSALRGNFNQAFATAGVAFLLEGFPEFTIPALGVFTFYSSIQEREKIIKTIENCLEQRVKRWKDSYQWMVSNWLSRITTQFNHINYQMYDSLSYQADAIKAKIDLEYKKYSGSDKENIKSQVENLKNSLDVKISEAMNNINKFIRECSVTYLFKNMLPKVIDELNKFDLRTKTELINLIDSHNIILVGEVDRLKAKVNESFENTMPFNIFSYTNNSLLKDIINEYFNSINDSKILSLQNKKNALVDTSGYNAEVRVGDNVQLNTIYTNDFKLSSSGDKIIVNLNNNILYSAIYENSSVSFWIKISKDLTNSHNEYTIINSIEQNSGWKLCIRNGNIEWILQDVNRKYKSLIFDYSESLSHTGYTNKWFFVTITNNIMGYMKLYINGELKQSQKIEDLDEVKLDKTIVFGIDENIDENQMLWIRDFNIFSKELSNEDINIVYEGQILRNVIKDYWGNPLKFDTEYYIINDNYIDRYIAPESNVLVLVQYPDRSKLYTGNPITIKSVSDKNPYSRILNGDNIILHMLYNSRKYMIIRDTDTIYATQGGECSQNCVYALKLQSNLGNYGIGIFSIKNIVSKNKYCSQIFSSFRENTMLLADIYKPWRFSFKNAYTPVAVTNYETKLLSTSSFWKFISRDPGWVE

SEQ ID NO: 21 - protein, 829 aa, synthetic construct
KSICIEINNGELFFVASENSYNDDNINTPKEIDDTVTSNNNYENDLDQVILNFNSESAPGLSDEKLNLTIQNDAYIPKYDSNGTSDIEQHDVNELNVFFYLDAQKVPEGENNVNLTSSIDTALLEQPKIYTFFSSEFINNVNKPVQAALFVGWIQQVLVDFTTEANQKSTVDKIADISIVVPYIGLALNIGNEAQKGNFKDALELLGAGILLEFEPELLIPTILVFTIKSFLGSSDNKNKVIKAINNALKERDEKWKEVYSFIVSNWMTKINTQFNKRKEQMYQALQNQVNALKAIIESKYNSYTLEEKNELTNKYDIEQIENELNQKVSIAMNNIDRFLTESSISYLMKLINEVKINKLREYDENVKTYLLDYIIKHGSILGESQQELNSMVIDTLNNSIPFKLSSYTDDKILISYFNKFFKRIKSSSVLNMRYKNDKYVDTSGYDSNININGDVYKYPTNKNQFGIYNDKLSEVNISQNDYIIYDNKYKNFSISFWVRIPNYDNKIVNVNNEYTIINCMRDNNSGWKVSLNHNEIIWTLQDNSGINQKLAFNYGNANGISDYINKWIFVTITNDRLGDSKLYINGNLIDKKSILNLGNIHVSDNILFKIVNCSYTRYIGIRYFNIFDKELDETEIQTLYNNEPNANILKDFWGNYLLYDKEYYLLNVLKPNNFINRRTDSTLSINNIRSTILLANRLYSGIKVKIQRVNNSSTNDNLVRKNDQVYINFVASKTHLLPLYADTATTNKEKTIKISSSGNRFNQVVVMNSVGNCTMNFKNNNGNNIGLLGFKADTVVASTWYYTHMRDNTNSNGFFWNFISEEHGWQEK

SEQ ID NO: 22 - protein, 835 aa, synthetic construct
APPRLCIRVNNSELFFVASESSYNENDINTPKEIDDTTNLNNNYRNNLDEVILDYNSQTIPQISNRTLNTLVQDNSYVPRYDSNGTSEIEEYDVVDFNVFFYLHAQKVPEGETNISLTSSIDTALLEESKDIFFSSEFIDTINKPVNAALFIDWISKVIRDFTTEATQKSTVDKIADISLIVPYVGLALNIIIEAEKGNFEEAFELLGVGILLEFVPELTIPVILVFTIKSYIDSYENKNKAIKAINNSLIEREAKWKEIYSWIVSNWLTRINTQFNKRKEQMYQALQNQVDAIKTAIEYKYNNYTSDEKNRLESEYNINNIEEELNKKVSLAMKNIERFMTESSISYLMKLINEAKVGKLKKYDNHVKSDLLNYILDHRSILGEQTNELSDLVTSTLNSSIPFELSSYTNDKILIIYFNRLYKKIKDSSILDMRYENNKFIDISGYGSNISINGNVYIYSTNRNQFGIYNSRLSEVNIAQNNDIIYNSRYQNFSISFWVRIPKHYKPMNHNREYTIINCMGNNNSGWKISLRTVRDCEIIWTLQDTSGNKENLIFRYEELNRISNYINKWIFVTITNNRLGNSRIYINGNLIVEKSISNLGDIHVSDNILFKIVGCDDETYVGIRYFKVFNTELDKTEIETLYSNEPDPSILKNYWGNYLLYNKKYYLFNLLRKDKYITLNSGILNINQQRGVTEGSVFLNYKLYEGVEVIIRKNGPIDISNTDNFVRKNDLAYINVVDRGVEYRLYADTKSEKEKIIRTSNLNDSLGQIIVMDSIGNNCTMNFQNNNGSNIGLLGFHSNNLVASSWYYNNIRRNTSSNGCFWSSISKENGWKE

SEQ ID NO: 23 - protein, 851 aa, synthetic construct
SEQCIIVNNEDLFFIANKDSFSKDLAKAETIAYNTQNNTIENNFSIDQLILDNDLSSGIDLPNENTEPFTNFDDIDIPVYIKQSALKKIFVDGDSLFEYLHAQTFPSNIENLQLTNSLNDALRNNNKVYTFFSTNLVEKANTVVGASLFVNWVKGVIDDFTSESTQKSTIDKVSDVSIIIPYIGPALNVGNETAKENFKNAFEIGGAAILMEFIPELIVPIVGFFTLESYVGNKGHIIMTISNALKKRDQKWTDMYGLIVSQWLSTVNTQFYTIKERMYNALNNQSQAIEKIIEDQYNRYSEEDKMNINIDFNDIDFKLNQSINLAINNIDDFINQCSISYLMNRMIPLAVKKLKDFDDNLKRDLLEYIDTNELYLLDEVNILKSKVNRHLKDSIPFDLSLYTKDTILIQVFNNYISNISSNAILSLSYRGGRLIDSSGYGATMNVGSDVIFNDIGNGQFKLNNSENSNITAHQSKFVVYDSMFDNFSINFWVRTPKYNNNDIQTYLQNEYTIISCIKNDSGWKVSIKGNRIIWTLIDVNAKSKSIFFEYSIKDNISDYINKWFSITITNDRLGNANIYINGSLKKSEKILNLDRINSSNDIDFKLINCTDTTKFVWIKDFNIFGRELNATEVSSLYWIQSSTNTLKDFWGNPLRYDTQYYLFNQGMQNIYIKYFSKASMGETAPRTNFNNAAINYQNLYLGLRFIIKKASNSRNINNDNIVREGDYIYLNIDNISDESYRVYVLVNSKEIQTQLFLAPINDDPTFYDVLQIKKYYEKTTYNCQILCEKDTKTFGLFGIGKFVKDYGYVWDTYDNYFCISQWYLRRISENINKLRLGCNWQFIPVDEGWTE

SEQ ID NO: 24 - protein, 18 aa, synthetic construct
MITETSSPFRSIFSHSGK

SEQ ID NO: 25 - protein, 8 aa, synthetic construct
HHHHHHHH

SEQ ID NO: 26 - protein, 238 aa, synthetic construct
VSKGEELFTGVVPILVELDGDVNGHKFSVRGEGEGDATNGKLTLKFICTTGKLPVPWPTLVTTLTYGVQCFSRYPDHMKQHDFFKSAMPEGYVQERTISFKDDGTYKTRAEVKFEGDTLVNRIELKGIDFKEDGNILGHKLEYNFNSHNVYITADKQKNGIKANFKIRHNVEDGSVQLADHYQQNTPIGDGPVLLPDNHYLSTQSKLSKDPNEKRDHMVLLEFVTAAGITLGMDELYK

SEQ ID NO: 27 - DNA, 39 bp, synthetic construct
  source 1..39: mol_type = other DNA
tacagatctagaatcgttgctttgaacgacttgtgtatc

SEQ ID NO: 28 - DNA, 40 bp, synthetic construct
  source 1..40: mol_type = other DNA
aacgattctagatctgtaagacttggtcttagaggtgatg

SEQ ID NO: 29 - DNA, 39 bp, synthetic construct
  source 1..39: mol_type = other DNA
aagcacttgtactctaacgctttgaacgacttgtgtatc

SEQ ID NO: 30 - DNA, 40 bp, synthetic construct
  source 1..40: mol_type = other DNA
gttagagtacaagtgcttagacttggtcttagaggtgatg

SEQ ID NO: 31 - DNA, 48 bp, synthetic construct
  source 1..48: mol_type = other DNA
gtttctcaagtttacccaatcgttcaagctttgaacgacttgtgtatc

SEQ ID NO: 32 - DNA, 40 bp, synthetic construct
  source 1..40: mol_type = other DNA
tgggtaaacttgagaaacagacttggtcttagaggtgatg

SEQ ID NO: 33 - DNA, 51 bp, synthetic construct
  source 1..51: mol_type = other DNA
ggtggttgggaacacgacggtatcgctttcgctttgaacgacttgtgtatc

SEQ ID NO: 34 - DNA, 37 bp, synthetic construct
  source 1..37: mol_type = other DNA
gtgttcccaaccaccagacttggtcttagaggtgatg

SEQ ID NO: 35 - DNA, 50 bp, synthetic construct
  source 1..50: mol_type = other DNA
ctcagacccagtctggtggttacagatctagaatcgttgctttgaacgac

SEQ ID NO: 36 - DNA, 40 bp, synthetic construct
  source 1..40: mol_type = other DNA
accagactgggtctgagaggtgatgatacctctaacacac

SEQ ID NO: 37 - DNA, 50 bp, synthetic construct
  source 1..50: mol_type = other DNA
ctcagacccagtctggtggtaagcacttgtactctaacgctttgaacgac

SEQ ID NO: 38 - DNA, 40 bp, synthetic construct; identical to SEQ ID NO: 36
  source 1..40: mol_type = other DNA

SEQ ID NO: 39 - DNA, 49 bp, synthetic construct
  source 1..49: mol_type = other DNA
ctcagacccagtctggtggtgtttctcaagtttacccaatcgttcaagc

SEQ ID NO: 40 - DNA, 40 bp, synthetic construct; identical to SEQ ID NO: 36
  source 1..40: mol_type = other DNA

SEQ ID NO: 41 - DNA, 29 bp, synthetic construct
  source 1..29: mol_type = other DNA
ctcagacccagtctggtggttgggaacac

SEQ ID NO: 42 - DNA, 40 bp, synthetic construct; identical to SEQ ID NO: 36
  source 1..40: mol_type = other DNA

SEQ ID NO: 43 - protein, 17 aa, synthetic construct
SNKTRIDEANQRATKML

SEQ ID NO: 44 - protein, 66 aa, synthetic construct
ARENEMDENLEQVSGIIGNLRHMALDMGNEIDTQNRQIDRIMEKADSNKTRIDEANQRATKMLGSG

SEQ ID NO: 45 - protein, 238 aa, synthetic construct
MSKGEELFTGVVPILVELDGDVNGHKFSVSGEGEGDATYGKLTLKFICTTGKLPVPWPTLVTTLTWGVQCFSRYPDHMKQHDFFKSAMPEGYVQERTIFFKDDGNYKTRAEVKFEGDTLVNRIELKGIDFKEDGNILGHKLEYNYISHNVYITADKQKNGIKANFKIRHNIEDGSVQLADHYQQNTPIGDGPVLLPDNHYLSTQSALSKDPNEKRDHMVLLEFVTAAGITHGMDELYK

SEQ ID NO: 46 - protein, 238 aa, synthetic construct
MSKGEELFTGVVPILVELDGDVNGHKFSVSGEGEGDATYGKLTLKFICTTGKLPVPWPTLVTTFGYGLQCFARYPDHMKRHDFFKSAMPEGYVQERTIFFKDDGNYKTRAEVKFEGDTLVNRIELKGIDFKEDGNILGHKLEYNYNSHNVYIMADKQKNGIKVNFKIRHNIEDGSVQLADHYQQNTPIGDGPVLLPDNHYLSYQSALSKDPNEKRDHMVLLEFVTAAGITHGMDELYK

SEQ ID NO: 47 - protein, 493 aa, synthetic construct
MSKGEELFTGVVPILVELDGDVNGHKFSVSGEGEGDATYGKLTLKFICTTGKLPVPWPTLVTTLTWGVQCFSRYPDHMKQHDFFKSAMPEGYVQERTIFFKDDGNYKTRAEVKFEGDTLVNRIELKGIDFKEDGNILGHKLEYNYISHNVYITADKQKNGIKANFKIRHNIEDGSVQLADHYQQNTPIGDGPVLLPDNHYLSTQSALSKDPNEKRDHMVLLEFVTAAGITHGMDELYKSNKTRIDEANQRATKMLMSKGEELFTGVVPILVELDGDVNGHKFSVSGEGEGDATYGKLTLKFICTTGKLPVPWPTLVTTFGYGLQCFARYPDHMKRHDFFKSAMPEGYVQERTIFFKDDGNYKTRAEVKFEGDTLVNRIELKGIDFKEDGNILGHKLEYNYNSHNVYIMADKQKNGIKVNFKIRHNIEDGSVQLADHYQQNTPIGDGPVLLPDNHYLSYQSALSKDPNEKRDHMVLLEFVTAAGITHGMDELYK

SEQ ID NO: 48 - protein, 542 aa, synthetic construct
MSKGEELFTGVVPILVELDGDVNGHKFSVSGEGEGDATYGKLTLKFICTTGKLPVPWPTLVTTLTWGVQCFSRYPDHMKQHDFFKSAMPEGYVQERTIFFKDDGNYKTRAEVKFEGDTLVNRIELKGIDFKEDGNILGHKLEYNYISHNVYITADKQKNGIKANFKIRHNIEDGSVQLADHYQQNTPIGDGPVLLPDNHYLSTQSALSKDPNEKRDHMVLLEFVTAAGITHGMDELYKARENEMDENLEQVSGIIGNLRHMALDMGNEIDTQNRQIDRIMEKADSNKTRIDEANQRATKMLGSGMSKGEELFTGVVPILVELDGDVNGHKFSVSGEGEGDATYGKLTLKFICTTGKLPVPWPTLVTTFGYGLQCFARYPDHMKRHDFFKSAMPEGYVQERTIFFKDDGNYKTRAEVKFEGDTLVNRIELKGIDFKEDGNILGHKLEYNYNSHNVYIMADKQKNGIKVNFKIRHNIEDGSVQLADHYQQNTPIGDGPVLLPDNHYLSYQSALSKDPNEKRDHMVLLEFVTAAGITHGMDELYK

SEQ ID NO: 49 - protein, 206 aa, synthetic construct
MAEDADMRNELEEMQRRADQLADESLESTRRMLQLVEESKDAGIRTLVMLDEQGEQLDRVEEGMNHINQDMKEAEKNLKDLGKCCGLFICPCNKLKSSDAYKKAWGNNQDGVVASQPARVVDEREQMAISGGFIRRVTNDARENEMDENLEQVSGIIGNLRHMALDMGNEIDTQNRQIDRIMEKADSNKTRIDEANQRATKMLGSG

SEQ ID NO: 50-51 - skipped (2 entries)